European Patent Application EP 4 382 128 A1, published June 12, 2024. Title: 一种增强核酸药物缓释能力的方法. Applicant: 成都凌泰氪生物技术有限公司. Application CN. The sequence listing filed with the application follows.

SEQUENCE LISTING (98 sequences)

SEQ ID NO: 1 - DNA, 19 bp, synthetic construct
  source 1..19: mol_type = other DNA
gggttgggtttgggttggg

SEQ ID NO: 2 - DNA, 80 bp, synthetic construct
  source 1..80: mol_type = other DNA
gctgtgtgactcctgcaaagtgtggacaacttcccacggaggaattcccgtatctaaaggtgcagctgtatcttgtctcc

SEQ ID NO: 3 - DNA, 118 bp, synthetic construct
  source 1..118: mol_type = other DNA
gctgtatcttgtctcctcagctgtgtgactcctgcaaagtgtggacaacttcccacggaggaattcccgtatctaaaggtgcagctgtatcttgtctccgctgtatcttgtctcctca

SEQ ID NO: 4 - DNA, 80 bp, synthetic construct; identical to SEQ ID NO: 2
  source 1..80: mol_type = other DNA

SEQ ID NO: 5 - DNA, 80 bp, synthetic construct
  source 1..80: mol_type = other DNA
ggagacaagatacagctgcacctttagatacgggaattcctccgtgggaagttgtccacactttgcaggagtcacacagc

SEQ ID NO: 6 - DNA, 118 bp, synthetic construct; identical to SEQ ID NO: 3
  source 1..118: mol_type = other DNA

SEQ ID NO: 7 - DNA, 118 bp, synthetic construct
  source 1..118: mol_type = other DNA
tgaggagacaagatacagcggagacaagatacagctgcacctttagatacgggaattcctccgtgggaagttgtccacactttgcaggagtcacacagctgaggagacaagatacagc

SEQ ID NO: 8 - RNA, 21 nt, synthetic construct
  source 1..21: mol_type = other RNA
ttgaatgtagagatgcggtgg

SEQ ID NO: 9 - RNA, 19 nt, synthetic construct
  source 1..19: mol_type = other RNA
gggttgggtttgggttggg

SEQ ID NO: 10 - RNA, 59 nt, synthetic construct
  source 1..59: mol_type = other RNA
gctgtatcttgtctcctcattgaatgtagagatgcggtgggctgtatcttgtctcctca

SEQ ID NO: 11 - RNA, 21 nt, synthetic construct
  source 1..21: mol_type = other RNA
ttgaatgtagagatgcggtgg

SEQ ID NO: 12 - RNA, 21 nt, synthetic construct
  source 1..21: mol_type = other RNA
ccaccgcatctctacattcaa

SEQ ID NO: 13 - RNA, 59 nt, synthetic construct; identical to SEQ ID NO: 10
  source 1..59: mol_type = other RNA

SEQ ID NO: 14 - RNA, 59 nt, synthetic construct
  source 1..59: mol_type = other RNA
tgaggagacaagatacagcccaccgcatctctacattcaatgaggagacaagatacagc

SEQ ID NO: 15 - DNA, 21 bp, synthetic construct
  source 1..21: mol_type = other DNA
ttgaatgtagagatgcggtgg

SEQ ID NO: 16 - DNA, 59 bp, synthetic construct
  source 1..59: mol_type = other DNA
gctgtatcttgtctcctcattgaatgtagagatgcggtgggctgtatcttgtctcctca

SEQ ID NO: 17 - DNA, 17 bp, synthetic construct
  source 1..17: mol_type = other DNA
gggtagggcgggttggg

SEQ ID NO: 18 - DNA, 19 bp, synthetic construct
  source 1..19: mol_type = other DNA
gggtttgggtgggtttggg

SEQ ID NO: 19 - DNA, 16 bp, synthetic construct
  source 1..16: mol_type = other DNA
gggtgggtgggtgggt

SEQ ID NO: 20 - DNA, 26 bp, synthetic construct
  source 1..26: mol_type = other DNA
ggtggtggtggttgtggtggtggtgg

SEQ ID NO: 21 - DNA, 28 bp, synthetic construct
  source 1..28: mol_type = other DNA
ggtggtggtggttgtttggtggtggtgg

SEQ ID NO: 22 - DNA, 24 bp, synthetic construct
  source 1..24: mol_type = other DNA
gtggggcattgtgggtgggtgtgg

SEQ ID NO: 23 - DNA, 22 bp, synthetic construct
  source 1..22: mol_type = other DNA
agggttagggttagggttaggg

SEQ ID NO: 24 - DNA, 15 bp, synthetic construct
  source 1..15: mol_type = other DNA
ggttggtgtggttgg

SEQ ID NO: 25 - DNA, 19 bp, synthetic construct
  source 1..19: mol_type = other DNA
gggtagggcggggttgggg

SEQ ID NO: 26 - DNA, 29 bp, synthetic construct
  source 1..29: mol_type = other DNA
ggtggtggtggttgtggtgggtgggtggg

SEQ ID NO: 27 - DNA, 53 bp, synthetic construct
  source 1..53: mol_type = other DNA
ggtggtggtggttgtggtggtggtggtggtggtggtggttgtggtggtggtgg

SEQ ID NO: 28 - DNA, 21 bp, synthetic construct
  source 1..21: mol_type = other DNA
ttgaatgtagagatgcggtgg

SEQ ID NO: 29 - DNA, 17 bp, synthetic construct
  source 1..17: mol_type = other DNA
gggaagggagggaaggg

SEQ ID NO: 30 - DNA, 17 bp, synthetic construct
  source 1..17: mol_type = other DNA
gggttgggtgggttggg

SEQ ID NO: 31 - DNA, 17 bp, synthetic construct
  source 1..17: mol_type = other DNA
gggccgggcgggccggg

SEQ ID NO: 32 - DNA, 18 bp, synthetic construct
  source 1..18: mol_type = other DNA
gggttgggttgggttggg

SEQ ID NO: 33 - DNA, 18 bp, synthetic construct
  source 1..18: mol_type = other DNA
gggtgggttttgggtggg

SEQ ID NO: 34 - DNA, 15 bp, synthetic construct
  source 1..15: mol_type = other DNA
gggtgggtgggtggg

SEQ ID NO: 35 - DNA, 16 bp, synthetic construct
  source 1..16: mol_type = other DNA
gggtgggttgggtggg

SEQ ID NO: 36 - DNA, 17 bp, synthetic construct
  source 1..17: mol_type = other DNA
gggtgggtttgggtggg

SEQ ID NO: 37 - DNA, 21 bp, synthetic construct
  source 1..21: mol_type = other DNA
gggtttgggtttgggtttggg

SEQ ID NO: 38 - DNA, 24 bp, synthetic construct
  source 1..24: mol_type = other DNA
gggttttgggttttgggttttggg

SEQ ID NO: 39 - DNA, 27 bp, synthetic construct
  source 1..27: mol_type = other DNA
gggtttttgggtttttgggtttttggg

SEQ ID NO: 40 - DNA, 23 bp, synthetic construct
  source 1..23: mol_type = other DNA
ggggttggggtttggggttgggg

SEQ ID NO: 41 - DNA, 27 bp, synthetic construct
  source 1..27: mol_type = other DNA
gggggttgggggtttgggggttggggg

SEQ ID NO: 42 - DNA, 31 bp, synthetic construct
  source 1..31: mol_type = other DNA
ggggggttggggggtttggggggttgggggg

SEQ ID NO: 43 - DNA, 35 bp, synthetic construct
  source 1..35: mol_type = other DNA
gggggggttgggggggtttgggggggttggggggg

SEQ ID NO: 44 - DNA, 39 bp, synthetic construct
  source 1..39: mol_type = other DNA
ggggggggttggggggggtttggggggggttgggggggg

SEQ ID NO: 45 - DNA, 43 bp, synthetic construct
  source 1..43: mol_type = other DNA
gggggggggttgggggggggtttgggggggggttggggggggg

SEQ ID NO: 46 - DNA, 47 bp, synthetic construct
  source 1..47: mol_type = other DNA
ggggggggggttggggggggggtttggggggggggttgggggggggg

SEQ ID NO: 47 - DNA, 22 bp, synthetic construct
  source 1..22: mol_type = other DNA
gggtagggcgggttgggtaggg

SEQ ID NO: 48 - DNA, 26 bp, synthetic construct
  source 1..26: mol_type = other DNA
gggtagggcgggttgggtagggcggg

SEQ ID NO: 49 - DNA, 31 bp, synthetic construct
  source 1..31: mol_type = other DNA
gggtagggcgggttgggtagggcgggttggg

SEQ ID NO: 50 - DNA, 34 bp, synthetic construct
  source 1..34: mol_type = other DNA
gggtagggcgggttggggggtagggcgggttggg

SEQ ID NO: 51 - DNA, 35 bp, synthetic construct
  source 1..35: mol_type = other DNA
gggtagggcgggttgggtgggtagggcgggttggg

SEQ ID NO: 52 - skipped

SEQ ID NO: 53 - DNA, 13 bp, synthetic construct
  source 1..13: mol_type = other DNA
attctagacattt

SEQ ID NO: 54 - DNA, 61 bp, synthetic construct
  source 1..61: mol_type = other DNA
ttgaatgtagagatgcggtgggggttgggtttgggttgggttgaatgtagagatgcggtgg

SEQ ID NO: 55 - DNA, 84 bp, synthetic construct
  source 1..84: mol_type = other DNA
tttgcctttaggagggttgggtttgggttgggttgaatgtagagatgcggtgggggttgggtttgggttgggttctagacattt

SEQ ID NO: 56 - RNA, 21 nt, synthetic construct
  source 1..21: mol_type = other RNA
ttgaatgtagagatgcggtgg

SEQ ID NO: 57 - DNA, 51 bp, synthetic construct
  source 1..51: mol_type = other DNA
gggttgggtttgggttggggtctgtggaagcggggttgggtttgggttggg

SEQ ID NO: 58 - DNA, 13 bp, synthetic construct
  source 1..13: mol_type = other DNA
gtctgtggaagcg

SEQ ID NO: 59 - DNA, 62 bp, synthetic construct
  source 1..62: mol_type = other DNA
gggttgggtttgggttgggagccacgtgggcagcagcctgtgagggttgggtttgggttggg

SEQ ID NO: 60 - DNA, 62 bp, synthetic construct
  source 1..62: mol_type = other DNA
gggttgggtttgggttgggttccacgtgggcagcagcctgtttgggttgggtttgggttggg

SEQ ID NO: 61 - DNA, 58 bp, synthetic construct
  source 1..58: mol_type = other DNA
gggttgggtttgggttgggcgtagacaccctcacccccagggttgggtttgggttggg

SEQ ID NO: 62 - DNA, 58 bp, synthetic construct
  source 1..58: mol_type = other DNA
gggttgggtttgggttgggtttagacaccctcaccccttgggttgggtttgggttggg

SEQ ID NO: 63 - DNA, 61 bp, synthetic construct
  source 1..61: mol_type = other DNA
gggttgggtttgggttgggtttagacaccctcacccccaattgggttgggtttgggttggg

SEQ ID NO: 64 - DNA, 61 bp, synthetic construct
  source 1..61: mol_type = other DNA
gggttgggtttgggttgggcgtagacaccctcacccccaaaagggttgggtttgggttggg

SEQ ID NO: 65 - DNA, 59 bp, synthetic construct
  source 1..59: mol_type = other DNA
gggttgggtttgggttgggttcatcccggccgctgaccttgggttgggtttgggttggg

SEQ ID NO: 66 - DNA, 56 bp, synthetic construct
  source 1..56: mol_type = other DNA
gggttgggtttgggttgggtttccccaaagtccccttgggttgggtttgggttggg

SEQ ID NO: 67 - DNA, 61 bp, synthetic construct
  source 1..61: mol_type = other DNA
gggttgggtttgggttgggttccacgtgggcagcagcctgttgggttgggtttgggttggg

SEQ ID NO: 68 - DNA, 62 bp, synthetic construct
  source 1..62: mol_type = other DNA
gggttgggtttgggttgggttgccacgtgggcagcagcctgttgggttgggtttgggttggg

SEQ ID NO: 69 - DNA, 56 bp, synthetic construct
  source 1..56: mol_type = other DNA
gggttgggtttgggttgggtttcagggaaccaggcttgggttgggtttgggttggg

SEQ ID NO: 70 - DNA, 56 bp, synthetic construct
  source 1..56: mol_type = other DNA
gggttgggtttgggttgggtttcctcagggaaccattgggttgggtttgggttggg

SEQ ID NO: 71 - DNA, 57 bp, synthetic construct
  source 1..57: mol_type = other DNA
gggttgggtttgggttgggttgctccggcagcagatttgggttgggtttgggttggg

SEQ ID NO: 72 - DNA, 56 bp, synthetic construct
  source 1..56: mol_type = other DNA
gggttgggtttgggttgggttgggatgctctgggcttgggttgggtttgggttggg

SEQ ID NO: 73 - DNA, 56 bp, synthetic construct
  source 1..56: mol_type = other DNA
gggttgggtttgggttgggttgcctgtctgtggaattgggttgggtttgggttggg

SEQ ID NO: 74 - DNA, 64 bp, synthetic construct
  source 1..64: mol_type = other DNA
gggttgggtttgggttgggttctggtcctcagggaaccaggccttgggttgggtttgggttggg

SEQ ID NO: 75 - DNA, 40 bp, synthetic construct
  source 1..40: mol_type = other DNA
cgggtttggctccgggtctggcgcgacctcatcctactca

SEQ ID NO: 76 - DNA, 62 bp, synthetic construct
  source 1..62: mol_type = other DNA
gggttgggtttgggttgggtttcgggtttggctccgggtctggcgcgacctcatcctactca

SEQ ID NO: 77 - DNA, 1617 bp, synthetic construct
  source 1..1617: mol_type = other DNA
gacattgattattgactagttattaatagtaatcaattacggggtcattagttcatagcccatatatggagttccgcgttacataacttacggtaaatggcccgcctggctgaccgcccaacgacccccgcccattgacgtcaataatgacgtatgttcccatagtaacgccaatagggactttccattgacgtcaatgggtggagtatttacggtaaactgcccacttggcagtacatcaagtgtatcatatgccaagtacgccccctattgacgtcaatgacggtaaatggcccgcctggcattatgcccagtacatgaccttatgggactttcctacttggcagtacatctacgtattagtcatcgctattaccatggtgatgcggttttggcagtacatcaatgggcgtggatagcggtttgactcacggggatttccaagtctccaccccattgacgtcaatgggagtttgttttggcaccaaaatcaacgggactttccaaaatgtcgtaacaactccgccccattgacgcaaatgggcggtaggcgtgtacggtgggaggtctatataagcagagctctctggctaactagagaacccactgcttactggcttatcgaaattaatacgactcactatagggagacccaagctggctagttaagcttcaccatggtgagcaagggcgaggagctgttcaccggggtggtgcccatcctggtcgagctggacggcgacgtaaacggccacaagttcagcgtgtccggcgagggcgagggcgatgccacctacggcaagctgaccctgaagttcatctgcaccaccggcaagctgcccgtgccctggcccaccctcgtgaccaccctgacctacggcgtgcagtgcttcagccgctaccccgaccacatgaagcagcacgacttcttcaagtccgccatgcccgaaggctacgtccaggagcgcaccatcttcttcaaggacgacggcaactacaagacccgcgccgaggtgaagttcgagggcgacaccctggtgaaccgcatcgagctgaagggcatcgacttcaaggaggacggcaacatcctggggcacaagctggagtacaactacaacagccacaacgtctatatcatggccgacaagcagaagaacggcatcaaggtgaacttcaagatccgccacaacatcgaggacggcagcgtgcagctcgccgaccactaccagcagaacacccccatcggcgacggccccgtgctgctgcccgacaaccactacctgagcacccagtccaagctgagcaaagaccccaacgagaagcgcgatcacatggtcctgctggagttcgtgaccgccgccgggatcactctcggcatggacgagctgtacaagtaataataaggatccagtacccttcaccaaagcaaaaatgtgatcttgcttgtaaatacaattttgagaggttaataaattacaagtagtgctatttttgtatttaggttagctatttagctttacgttccaggatgcctagtggcagccccacaatatccaggaagccctctctgcggtttttcagattaggtagtcgaaaaacctaagaaatttacctgct

SEQ ID NO: 78 - DNA, 1655 bp, synthetic construct
  source 1..1655: mol_type = other DNA
gggttgggtttgggttggggacattgattattgactagttattaatagtaatcaattacggggtcattagttcatagcccatatatggagttccgcgttacataacttacggtaaatggcccgcctggctgaccgcccaacgacccccgcccattgacgtcaataatgacgtatgttcccatagtaacgccaatagggactttccattgacgtcaatgggtggagtatttacggtaaactgcccacttggcagtacatcaagtgtatcatatgccaagtacgccccctattgacgtcaatgacggtaaatggcccgcctggcattatgcccagtacatgaccttatgggactttcctacttggcagtacatctacgtattagtcatcgctattaccatggtgatgcggttttggcagtacatcaatgggcgtggatagcggtttgactcacggggatttccaagtctccaccccattgacgtcaatgggagtttgttttggcaccaaaatcaacgggactttccaaaatgtcgtaacaactccgccccattgacgcaaatgggcggtaggcgtgtacggtgggaggtctatataagcagagctctctggctaactagagaacccactgcttactggcttatcgaaattaatacgactcactatagggagacccaagctggctagttaagcttcaccatggtgagcaagggcgaggagctgttcaccggggtggtgcccatcctggtcgagctggacggcgacgtaaacggccacaagttcagcgtgtccggcgagggcgagggcgatgccacctacggcaagctgaccctgaagttcatctgcaccaccggcaagctgcccgtgccctggcccaccctcgtgaccaccctgacctacggcgtgcagtgcttcagccgctaccccgaccacatgaagcagcacgacttcttcaagtccgccatgcccgaaggctacgtccaggagcgcaccatcttcttcaaggacgacggcaactacaagacccgcgccgaggtgaagttcgagggcgacaccctggtgaaccgcatcgagctgaagggcatcgacttcaaggaggacggcaacatcctggggcacaagctggagtacaactacaacagccacaacgtctatatcatggccgacaagcagaagaacggcatcaaggtgaacttcaagatccgccacaacatcgaggacggcagcgtgcagctcgccgaccactaccagcagaacacccccatcggcgacggccccgtgctgctgcccgacaaccactacctgagcacccagtccaagctgagcaaagaccccaacgagaagcgcgatcacatggtcctgctggagttcgtgaccgccgccgggatcactctcggcatggacgagctgtacaagtaataataaggatccagtacccttcaccaaagcaaaaatgtgatcttgcttgtaaatacaattttgagaggttaataaattacaagtagtgctatttttgtatttaggttagctatttagctttacgttccaggatgcctagtggcagccccacaatatccaggaagccctctctgcggtttttcagattaggtagtcgaaaaacctaagaaatttacctgctgggttgggtttgggttggg

SEQ ID NO: 79 - RNA, 2394 nt, synthetic construct
  source 1..2394: mol_type = other RNA
ttaaaacagcctgtgggttgatcccacccacaggcccattgggcgctagcactctggtatcacggtacctttgtgcgcctgttttataccccctcccccaactgtaacttagaagtaacacacaccgatcaacagtcagcgtggcacaccagccacgttttgatcaagcacttctgttaccccggactgagtatcaatagactgctcacgcggttgaaggagaaagcgttcgttatccggccaactacttcgaaaaacctagtaacaccgtggaagttgcagagtgtttcgctcagcactaccccagtgtagatcaggtcgatgagtcaccgcattccccacgggcgaccgtggcggtggctgcgttggcggcctgcccatggggaaacccatgggacgctctaatacagacatggtgcgaagagtctattgagctagttggtagtcctccggcccctgaatgcggctaatcctaactgcggagcacacaccctcaagccagagggcagtgtgtcgtaacgggcaactctgcagcggaaccgactactttgggtgtccgtgtttcattttattcctatactggctgcttatggtgacaattgagagatcgttaccatatagctattggattggccatccggtgactaatagagctattatatatccctttgttgggtttataccacttagcttgaaagaggttaaaacattacaattcattgttaagttgaatacagcaaaatggccgatgctaagaacattaagaagggccctgctcccttctaccctctggaggatggcaccgctggcgagcagctgcacaaggccatgaagaggtatgccctggtgcctggcaccattgccttcaccgatgcccacattgaggtggacatcacctatgccgagtacttcgagatgtctgtgcgcctggccgaggccatgaagaggtacggcctgaacaccaaccaccgcatcgtggtgtgctctgagaactctctgcagttcttcatgccagtgctgggcgccctgttcatcggagtggccgtggcccctgctaacgacatttacaacgagcgcgagctgctgaacagcatgggcatttctcagcctaccgtggtgttcgtgtctaagaagggcctgcagaagatcctgaacgtgcagaagaagctgcctatcatccagaagatcatcatcatggactctaagaccgactaccagggcttccagagcatgtacacattcgtgacatctcatctgcctcctggcttcaacgagtacgacttcgtgccagagtctttcgacagggacaaaaccattgccctgatcatgaacagctctgggtctaccggcctgcctaagggcgtggccctgcctcatcgcaccgcctgtgtgcgcttctctcacgcccgcgaccctattttcggcaaccagatcatccccgacaccgctattctgagcgtggtgccattccaccacggcttcggcatgttcaccaccctgggctacctgatttgcggctttcgggtggtgctgatgtaccgcttcgaggaggagctgttcctgcgcagcctgcaagactacaaaattcagtctgccctgctggtgccaaccctgttcagcttcttcgctaagagcaccctgatcgacaagtacgacctgtctaacctgcacgagattgcctctggcggcgccccactgtctaaggaggtgggcgaagccgtggccaagcgctttcatctgccaggcatccgccagggctacggcctgaccgagacaaccagcgccattctgattaccccagagggcgacgacaagcctggcgccgtgggcaaggtggtgccattcttcgaggccaaggtggtggacctggacaccggcaagaccctgggagtgaaccagcgcggcgagctgtgtgtgcgcggccctatgattatgtccggctacgtgaataaccctgaggccacaaacgccctgatcgacaaggacggctggctgcactctggcgacattgcctactgggacgaggacgagcacttcttcatcgtggaccgcctgaagtctctgatcaagtacaagggctaccaggtggccccagccgagctggagtctatcctgctgcagcaccctaacattttcgacgccggagtggccggcctgcccgacgacgatgccggcgagctgcctgccgccgtcgtcgtgctggaacacggcaagaccatgaccgagaaggagatcgtggactatgtggccagccaggtgacaaccgccaagaagctgcgcggcggagtggtgttcgtggacgaggtgcccaagggcctgaccggcaagctggacgcccgcaagatccgcgagatcctgatcaaggctaagaaaggcggcaagatcgccgtgtaa

SEQ ID NO: 80 - RNA, 2432 nt, synthetic construct
  source 1..2432: mol_type = other RNA
gggttgggtttgggttgggttaaaacagcctgtgggttgatcccacccacaggcccattgggcgctagcactctggtatcacggtacctttgtgcgcctgttttataccccctcccccaactgtaacttagaagtaacacacaccgatcaacagtcagcgtggcacaccagccacgttttgatcaagcacttctgttaccccggactgagtatcaatagactgctcacgcggttgaaggagaaagcgttcgttatccggccaactacttcgaaaaacctagtaacaccgtggaagttgcagagtgtttcgctcagcactaccccagtgtagatcaggtcgatgagtcaccgcattccccacgggcgaccgtggcggtggctgcgttggcggcctgcccatggggaaacccatgggacgctctaatacagacatggtgcgaagagtctattgagctagttggtagtcctccggcccctgaatgcggctaatcctaactgcggagcacacaccctcaagccagagggcagtgtgtcgtaacgggcaactctgcagcggaaccgactactttgggtgtccgtgtttcattttattcctatactggctgcttatggtgacaattgagagatcgttaccatatagctattggattggccatccggtgactaatagagctattatatatccctttgttgggtttataccacttagcttgaaagaggttaaaacattacaattcattgttaagttgaatacagcaaaatggccgatgctaagaacattaagaagggccctgctcccttctaccctctggaggatggcaccgctggcgagcagctgcacaaggccatgaagaggtatgccctggtgcctggcaccattgccttcaccgatgcccacattgaggtggacatcacctatgccgagtacttcgagatgtctgtgcgcctggccgaggccatgaagaggtacggcctgaacaccaaccaccgcatcgtggtgtgctctgagaactctctgcagttcttcatgccagtgctgggcgccctgttcatcggagtggccgtggcccctgctaacgacatttacaacgagcgcgagctgctgaacagcatgggcatttctcagcctaccgtggtgttcgtgtctaagaagggcctgcagaagatcctgaacgtgcagaagaagctgcctatcatccagaagatcatcatcatggactctaagaccgactaccagggcttccagagcatgtacacattcgtgacatctcatctgcctcctggcttcaacgagtacgacttcgtgccagagtctttcgacagggacaaaaccattgccctgatcatgaacagctctgggtctaccggcctgcctaagggcgtggccctgcctcatcgcaccgcctgtgtgcgcttctctcacgcccgcgaccctattttcggcaaccagatcatccccgacaccgctattctgagcgtggtgccattccaccacggcttcggcatgttcaccaccctgggctacctgatttgcggctttcgggtggtgctgatgtaccgcttcgaggaggagctgttcctgcgcagcctgcaagactacaaaattcagtctgccctgctggtgccaaccctgttcagcttcttcgctaagagcaccctgatcgacaagtacgacctgtctaacctgcacgagattgcctctggcggcgccccactgtctaaggaggtgggcgaagccgtggccaagcgctttcatctgccaggcatccgccagggctacggcctgaccgagacaaccagcgccattctgattaccccagagggcgacgacaagcctggcgccgtgggcaaggtggtgccattcttcgaggccaaggtggtggacctggacaccggcaagaccctgggagtgaaccagcgcggcgagctgtgtgtgcgcggccctatgattatgtccggctacgtgaataaccctgaggccacaaacgccctgatcgacaaggacggctggctgcactctggcgacattgcctactgggacgaggacgagcacttcttcatcgtggaccgcctgaagtctctgatcaagtacaagggctaccaggtggccccagccgagctggagtctatcctgctgcagcaccctaacattttcgacgccggagtggccggcctgcccgacgacgatgccggcgagctgcctgccgccgtcgtcgtgctggaacacggcaagaccatgaccgagaaggagatcgtggactatgtggccagccaggtgacaaccgccaagaagctgcgcggcggagtggtgttcgtggacgaggtgcccaagggcctgaccggcaagctggacgcccgcaagatccgcgagatcctgatcaaggctaagaaaggcggcaagatcgccgtgtaagggttgggtttgggttggg

SEQ ID NO: 81 - RNA, 1019 nt, synthetic construct
  source 1..1019: mol_type = other RNA
ttagcagtaactgctgaattcctggttggctgatggaaagatggggcagctgttcactggtacgcagggttttagatgtatgtacctaaggatatgaggtatggcaatgaacagaaattcttttgggaatgagttttagggccattaaaggacatgacctgaagtttcctctgaggccagtccccacaactcaatataaatgtgtttcctgcatatagtcaaagttgccacttctttttcttcatatcatcgatctctgctcttaaagataatcttggttttgcctcaaactgtttgtcactacaaactttccccatgttcctaagtaaaacaggtaactgcctctcaactatatcaagtagactaaaatattgtgtctctaatatcagaaattcagctttaatatattgggtttaactctttgaaatttagagtctccttgaaatacacatgggggtgatttcctaaactttatttcttgtaaggatttatctcaggggtaacacacaaaccagcatcctgaacctctaagtatgaggacagtaagccttaagaatataaaataaactgttcttctctctgccggtggaagtgtgccctgtctattcctgaaattgcttgtttgagacgcatgagacgtgcagcacatgagacacgtgcagcagcctgtggaatattgtcagtgaagaatgtctttgcctgattagatataaagacaagttaaacacagcattagactatagatcaagcctgtgccagacacaaatgacctaatgcccagcacgggccacggaatctcctatcctcttgcttgaacagagcagcacacttctcccccaacactattagatgttctggcataattttgtagatatgtaggatttgacatggactattgttcaatgattcagaggaaatctcctttgttcagataagtacactgactactaaatggattaaaaaacacagtaataaaacccagttttccccttaaaaaaaaaaaaaaaaaaaaaaaaaaa

SEQ ID NO: 82 - RNA, 1057 nt, synthetic construct
  source 1..1057: mol_type = other RNA
gggttgggtttgggttgggttagcagtaactgctgaattcctggttggctgatggaaagatggggcagctgttcactggtacgcagggttttagatgtatgtacctaaggatatgaggtatggcaatgaacagaaattcttttgggaatgagttttagggccattaaaggacatgacctgaagtttcctctgaggccagtccccacaactcaatataaatgtgtttcctgcatatagtcaaagttgccacttctttttcttcatatcatcgatctctgctcttaaagataatcttggttttgcctcaaactgtttgtcactacaaactttccccatgttcctaagtaaaacaggtaactgcctctcaactatatcaagtagactaaaatattgtgtctctaatatcagaaattcagctttaatatattgggtttaactctttgaaatttagagtctccttgaaatacacatgggggtgatttcctaaactttatttcttgtaaggatttatctcaggggtaacacacaaaccagcatcctgaacctctaagtatgaggacagtaagccttaagaatataaaataaactgttcttctctctgccggtggaagtgtgccctgtctattcctgaaattgcttgtttgagacgcatgagacgtgcagcacatgagacacgtgcagcagcctgtggaatattgtcagtgaagaatgtctttgcctgattagatataaagacaagttaaacacagcattagactatagatcaagcctgtgccagacacaaatgacctaatgcccagcacgggccacggaatctcctatcctcttgcttgaacagagcagcacacttctcccccaacactattagatgttctggcataattttgtagatatgtaggatttgacatggactattgttcaatgattcagaggaaatctcctttgttcagataagtacactgactactaaatggattaaaaaacacagtaataaaacccagttttccccttaaaaaaaaaaaaaaaaaaaaaaaaaaagggttgggtttgggttggg

SEQ ID NO: 83 - DNA, 24 bp, synthetic construct
  source 1..24: mol_type = other DNA
agccacgtgggcagcagcctgtga

SEQ ID NO: 84 - DNA, 24 bp, synthetic construct
  source 1..24: mol_type = other DNA
ttccacgtgggcagcagcctgttt

SEQ ID NO: 85 - DNA, 20 bp, synthetic construct
  source 1..20: mol_type = other DNA
cgtagacaccctcaccccca

SEQ ID NO: 86 - DNA, 20 bp, synthetic construct
  source 1..20: mol_type = other DNA
tttagacaccctcacccctt

SEQ ID NO: 87 - DNA, 23 bp, synthetic construct
  source 1..23: mol_type = other DNA
tttagacaccctcacccccaatt

SEQ ID NO: 88 - DNA, 23 bp, synthetic construct
  source 1..23: mol_type = other DNA
cgtagacaccctcacccccaaaa

SEQ ID NO: 89 - DNA, 21 bp, synthetic construct
  source 1..21: mol_type = other DNA
ttcatcccggccgctgacctt

SEQ ID NO: 90 - DNA, 18 bp, synthetic construct
  source 1..18: mol_type = other DNA
tttccccaaagtcccctt

SEQ ID NO: 91 - DNA, 23 bp, synthetic construct
  source 1..23: mol_type = other DNA
ttccacgtgggcagcagcctgtt

SEQ ID NO: 92 - DNA, 24 bp, synthetic construct
  source 1..24: mol_type = other DNA
ttgccacgtgggcagcagcctgtt

SEQ ID NO: 93 - DNA, 18 bp, synthetic construct
  source 1..18: mol_type = other DNA
tttcagggaaccaggctt

SEQ ID NO: 94 - DNA, 18 bp, synthetic construct
  source 1..18: mol_type = other DNA
tttcctcagggaaccatt

SEQ ID NO: 95 - DNA, 19 bp, synthetic construct
  source 1..19: mol_type = other DNA
ttgctccggcagcagattt

SEQ ID NO: 96 - DNA, 18 bp, synthetic construct
  source 1..18: mol_type = other DNA
ttgggatgctctgggctt

SEQ ID NO: 97 - DNA, 18 bp, synthetic construct
  source 1..18: mol_type = other DNA
ttgcctgtctgtggaatt

SEQ ID NO: 98 - DNA, 26 bp, synthetic construct
  source 1..26: mol_type = other DNA
ttctggtcctcagggaaccaggcctt